European Patent Application EP 4 116 425 A1, published January 11, 2023. Title: GENETICALLY MODIFIED BACTERIA AND USES THEREOF FOR THE INDUCIBLE EXPRESSION OF A NUCLEIC SEQUENCE OF INTEREST. Applicant: Institut national de recherche pour l'agriculture, l'alimentation et l'environnement Institut des sciences et industries du vivant et de l'environnement. The sequence listing filed with the application follows.

SEQUENCE LISTING (45 sequences)

SEQ ID NO: 1 - DNA, 15 bp, Streptococcus thermophilus
  misc_feature (4)..(4): W = A or T
  misc_feature (8)..(8): K = T or G
  misc_feature (15)..(15): W = A or T
gcawatakgggaatw

SEQ ID NO: 2 - DNA, 18 bp, Streptococcus thermophilus
  misc_feature (7)..(7): K = G or T
aattgcktataagggaaa

SEQ ID NO: 3 - DNA, 19 bp, Streptococcus thermophilus
atttcatatcttcaatttt

SEQ ID NO: 4 - protein, 285 aa, Streptococcus thermophilus
MKDYGKLFKKFRESRGLVLKDIAKLGVSVSHISRFERENTDLTISKFMSALNAINMPIDEFMYAANDFQRDEFNEILEKISLFVSARNVSGMEKLLISQVEKIEKRETFYTLNTILIKIRLQDLSDKSYYDESDIQYLSDYLFSVEYWGCYELLLFANTVDVLNHQTMMLLSREMCKRSEFYKDLPNYRRLHSTMLLNCYIISIERDEYIDALYFEKQLNHSCFTETEIYEKLVFHYSKNLYELKKNRSNKAILEMKKCITAMKLANSENLAIKFENHLSGVLKM

SEQ ID NO: 5 - protein, 291 aa, Streptococcus thermophilus
MDSNELLKLGEFYKELRIARKVKQKDVAKNKLSVSQLSKFESGQTMLSADKMLEVIEGINLTFSEFGFALRDYKPTQHQLLMNKISKLSAENDKQSLLKLLDKYKESQLLYDKLNTLVIKNAIHLIDRDFTLSLDDSKFLSNYLFDIEDWTAYEIHLFGNTMPFLSDTDLLFLGKELVSRSEIYSPLLDFRKALKYTYLNLISELVERRLTTHFNFFVNQLRMILDVFDTFEIILLNFLVLVYSYLIENSVNLEEVEQYILKVSEIEQLGLSKILEQRLSQYLRTNQKGER

SEQ ID NO: 6 - protein, 286 aa, Streptococcus thermophilus
MKKFGEIFKKFRESRGLRLKDVAKAGISTSQLSRFEKGETDLTISKFMFILDEINMPIDEFMYAVHDFHRDELNELLSKVRHFVSTRDVEGMKKLLYSQMELEDRREKFHQINIILLKIRLQDLSGETYYTKDDLTYLTDYLFSVEYWGYYELLIFSNTLDVLNHDVFMVLAREMFRRSDFYKEIPNNRRLISTMLLNGYITCVEREKFMDALYFEKQLNQCFFIETEVYERLVFKYAQNLYQYKEDGNVKAIIEMKKCVGAMKLAGSHHLAKTYEGHLEKILASS

SEQ ID NO: 7 - protein, 287 aa, Streptococcus thermophilus
MKEFGAIFKKFRKSRGIRLKDVAKAGISTSQLSRFEKGQTDLTITKFMLILDEINMPIDEFMYAVHDFHRDDLNELLSKIRLFVSTHDIDGLKKLLSSQLESEPKREKFHHINTILLKIRLQDLSGESYYTQQDLADLTDYLFSVEYWGYYELLIFANTLDVLNHETLMVLAKEMSRRSDFYKEIPNNRRMISTMLLNVYITCIEREELIDALYFEKQLNQCFFIETEIYERLVFQYAQNYYQYKKEGNNQSIIEMKKYIGAMKLAGSEHIAKTYEAHLKKLIEENS

SEQ ID NO: 8 - protein, 232 aa, Streptococcus thermophilus
MPIEEFVYAVRDFRRDDFNELLEKIRYLVSNRDIDGMKKLLISQMEKKDKKEPFASFNTILIKIRLQDLSGETYVTDQEIVTISDYLFSAEYWGYYELLLFMNTIDALNHNTMMILAKEMCHRLDFYRDIPNNRRLLATMLLNAYITCIERNEWMDALYFEKQLKYCNFSETEMYEKLVLHYANNLYDLKKNNNRHAVLEMRKCIAATKLVDSNQISIKFENYLQKVLDDMR

SEQ ID NO: 9 - protein, 238 aa, Streptococcus thermophilus
MIKFLSALDFINVSIEEFMVIYRGYRNDSFEELLKKLHTLSLTKDAEGLRYLFNEVEELPNSTTKKIEKILILSCLSSVESENLITQSDLRFVTDYLFGIESWGYYELSILGNLAQYINGETLVSLGREVLRKTDYYYEVVRNRKLVIQLSINIMIRCIESEWFTKAAFFERHIDSLVNVESDMYEKVIFSYVQGYLKFAMGDSGGKQIMQESLEIFKLLKNTRLYKNYLEHFKSIVG

SEQ ID NO: 10 - protein, 284 aa, Streptococcus thermophilus
MKSKLGSTLRKVRNGKQISICSVADEHLSKSQISRFERGESEISCIRLINILDKLHITLDEFLILHDEDYTKTESFANLVQYIRKQYSLQNINNIQSLLSDSSNYTLDPFEKTMVKSILHTMDSSIIPSDDELLQLADYLFKVEKWGYYEIILLGNCVRTIDYNSVFLLTKEMLNNYIYSSLNKTNKRIVTQLAINCLILSIDMEEFTNCFYLIDEIKALLDNELNFYEQTVFLYATGYFEFKRWQSTSGIEKMKQAIQVLDILGEDNLKLHYTIHFDKLINNK

SEQ ID NO: 11 - protein, 287 aa, Streptococcus thermophilus
MNIQEKFKAIRKQRKLSLRDLANVAGSTSSISDFEKGKTNLSNDVLLQLLGFMVVEINEIFEWSAFQDAEFLELMTQVENALQTQDITVLIQKRETLQEFFVAKNHYIYHIISLVLDVIISKLQEKEPTPEIISELTDYFFSLDYWTNLDVGLLGNIVHHFTTETLVLFTDSILKNTPNQLRNNLDRIKIDTVINCLSVLLARREKNASQELLQLLSRKQFPTYFTYEKLCISEFKAIYMYIWCDKEEADNIHQTILKTVSLLFTKDEANKWDDYFKEIISSADIKK

SEQ ID NO: 12 - protein, 286 aa, Streptococcus thermophilus
MNTNESMDLGELFRELRIARGLKLKDVASDKLSVSQLSKFENGQTMLSSDKLLVAISGIHMNFSEFGYALNNYQEPEFFKLGEKIAALHSKQDIDGLKKLLVTYKGCESFDVYNRLNLLVIKVAIHSLDNSSLITDEDKEFLTNYLYEIEAWTEYELYIFGNTMSILSDSDLIFLGKAFEERSKLYSSLTSHKKSAEIAFLNLILILIERKEIYYVRYFMSKLEEILNYQDMFAITYLHVLKQVSDYLNGDVKSIEKIDNDINMIEKLGNPIAASFLRINLQQFLH

SEQ ID NO: 13 - protein, 290 aa, Streptococcus thermophilus
MLTKFGEIYKLFRESRKITLRDIEHRGISRSQLSRFEKGETDLTTTKFFLALEQINVPIEEFMYAVKDFKRDCFYQLIDEVKQCFLNRNVPKLHKMLIKRMENDDTSIFSTIEIIFLKIKLQELSGEEYFNDTDINRITDYLFGVNYWGMFEILLFGNIMYIFNYETFLLLSKELLHRTEFYHDIPSYRRVIASIALNAFIICIERDYLVDAKYFEKQISRFYFDESEIYERLIYTYARSFYEFKKKQTTQSILKMRKVIGFMRVVECEKLAERYEEHLNKILSSFSDDN

SEQ ID NO: 14 - DNA, 15 bp, Streptococcus thermophilus
gcaaataggggaata

SEQ ID NO: 15 - DNA, 15 bp, Streptococcus thermophilus
gcaaataggggaatt

SEQ ID NO: 16 - DNA, 15 bp, Streptococcus thermophilus
gcatataggggaata

SEQ ID NO: 17 - DNA, 15 bp, Streptococcus thermophilus
gcatataggggaatt

SEQ ID NO: 18 - DNA, 15 bp, Streptococcus thermophilus
gcaaatatgggaata

SEQ ID NO: 19 - DNA, 15 bp, Streptococcus thermophilus
gcaaatatgggaatt

SEQ ID NO: 20 - DNA, 15 bp, Streptococcus thermophilus
gcatatatgggaata

SEQ ID NO: 21 - DNA, 15 bp, Streptococcus thermophilus
gcatatatgggaatt

SEQ ID NO: 22 - DNA, 18 bp, Streptococcus thermophilus
aattgcgtataagggaaa

SEQ ID NO: 23 - DNA, 18 bp, Streptococcus thermophilus
aattgcttataagggaaa

SEQ ID NO: 24 - protein, 9 aa, Streptococcus thermophilus
EGIIVIVVG

SEQ ID NO: 25 - protein, 9 aa, Streptococcus thermophilus
EGIIVILVG

SEQ ID NO: 26 - protein, 9 aa, Streptococcus thermophilus
EGIIVIGVG

SEQ ID NO: 27 - protein, 9 aa, Streptococcus thermophilus
ESIIVIAVG

SEQ ID NO: 28 - protein, 9 aa, Streptococcus thermophilus
DIIIFPPFG

SEQ ID NO: 29 - protein, 8 aa, Streptococcus thermophilus
DIIIIVGG

SEQ ID NO: 30 - protein, 8 aa, Streptococcus thermophilus
EIIIIIAL

SEQ ID NO: 31 - protein, 9 aa, Streptococcus thermophilus
CIYTIVGGV

SEQ ID NO: 32 - protein, 9 aa, Streptococcus thermophilus
CIYIIVGGV

SEQ ID NO: 33 - protein, 23 aa, Streptococcus thermophilus
MKKQILLTLLLVVFEGIIVIVVG

SEQ ID NO: 34 - protein, 23 aa, Streptococcus thermophilus
MKKQKLLLLVVLVCEGIIVILVG

SEQ ID NO: 35 - protein, 23 aa, Streptococcus thermophilus
MNKKALFSLLFVILEGIIVIGVG

SEQ ID NO: 36 - protein, 23 aa, Streptococcus thermophilus
MNKESFLAILLLIFESIIVIAVG

SEQ ID NO: 37 - protein, 26 aa, Streptococcus thermophilus
MKKVIAIFLFIQTVVVIDIIIFPPFG

SEQ ID NO: 38 - protein, 23 aa, Streptococcus thermophilus
MEKVSKILPILILVMDIIIIVGG

SEQ ID NO: 39 - protein, 21 aa, Streptococcus thermophilus
MNISIKRFLMILLEIIIIIAL

SEQ ID NO: 40 - protein, 20 aa, Streptococcus thermophilus
MKLLKIIVLLTCIYTIVGGV

SEQ ID NO: 41 - protein, 20 aa, Streptococcus thermophilus
MKLLKIIVLLTCIYIIVGGV

SEQ ID NO: 42 - protein, 243 aa, Streptococcus thermophilus
MLKLEKVTGGYANIPVLKDVTFEVADGELVGLIGLNGAGKSTTINEIIGLLTPYGGQIAIDGLTIQQDPASYRQKIGYIPETPSLYEELTLREHLETVLMAYGLDVTEGMARADKYLKLFRLDEKLDWFPTQFSKGMKQKVMIICAFIVNPSLFIVDEPFLGLDPLAISDLIELLAEEKANGKSILMSTHVLDSAEKMCDRFVILHHGQILAQGTIDELRQTFGDSSASLNDIYMQLTKGELS

SEQ ID NO: 43 - protein, 345 aa, Streptococcus thermophilus
MIAELFKERSRRLTTRCAKYSRYVFNDHFILVLLFLLGFVLVQYSQLLRHFPKNPWAIILGLLVLCLLLPFWGNIATYLEPADKHYLLVKEEEVLDHIKKATGCAFRFWVLIQTLIFILVVPLFLALGLPVWGVVLVAVAMAILKYFIFQKKAQPFYKQSGLNWTDAIAAENKRQQSILKFFSLFTNVKGITSSVKRRGYLDGILKRTKKDKKYTWYNLYLRAFLRSGDYFALSLRLFALTLLVIFLVPEKWLAMVLVVVFDYLLLFQLTALKSHFAYQRMANLMPIGKDMQVSNLKRLINQIVLVMTLIQALCLFDLKFSLILIGVMLVLSLVYLPAKLKKMID

SEQ ID NO: 44 - protein, 420 aa, Streptococcus thermophilus
MKAIITFLLIFCVIVVFHEFGHFFFAKRSGILVREFAIGMGPKIFAHTGKDGTVYTIRILPLGGYVRMAGWGEDTTEIKTGSPASLTLGKDGKVRRINLSDRQVDQTALPMNVTAYDLEDKLTITGLVLGETKTYEVDHDATIVEEDGTELRIAPKDVQYQNASIWGRLITNFAGPMNNFILGVLVFIILAFVQGGVQDTSTNLIQVTNGGAAQVSGLKTGDAIVAINKDKVTDWDSLKEALRENTQKFSKGDSLSVTVKRSNGQEETISVKPQESQGSYFLGVSPVLKTGLKDKIFGGFQMAWEGATAILATLKGLITNFSLNKLGGPVAMFQMSAQASESGLISILDLMGMLSINLGIFNLIPIPALDGGKIVMNIIEAIRRKPLNQKIESYITLAGVAVMVVLMIAVTWNDIMRAFF

SEQ ID NO: 45 - protein, 8 aa, artificial sequence
  Synthetic peptide
LPYFAGCL